European Patent Specification EP 4 448 794 B1, published January 21, 2026. Title: COMPOSITIONS, KITS, AND METHODS FOR SHORT TANDEM REPEAT ANALYSIS. Applicant: Life Technologies Corporation. The sequence listing filed with the application follows.

SEQUENCE LISTING (192 sequences)

SEQ ID NO: 1 - DNA, 20 bp, synthetic construct
  misc_feature 1..20: note = Synthetic oligonucleotide
  source 1..20: mol_type = other DNA
aacaagagcctgggacctcc

SEQ ID NO: 2 - DNA, 20 bp, synthetic construct
  misc_feature 1..20: note = Synthetic oligonucleotide
  source 1..20: mol_type = other DNA
gcagaaggtgaaggggagca

SEQ ID NO: 3 - DNA, 21 bp, synthetic construct
  misc_feature 1..21: note = Synthetic oligonucleotide
  source 1..21: mol_type = other DNA
agctctgccctcatgaatgct

SEQ ID NO: 4 - DNA, 20 bp, synthetic construct
  misc_feature 1..20: note = Synthetic oligonucleotide
  source 1..20: mol_type = other DNA
tcatgaaccgcctctcacga

SEQ ID NO: 5 - DNA, 20 bp, synthetic construct
  misc_feature 1..20: note = Synthetic oligonucleotide
  source 1..20: mol_type = other DNA
aatggcgtgaacccgggaag

SEQ ID NO: 6 - DNA, 19 bp, synthetic construct
  misc_feature 1..19: note = Synthetic oligonucleotide
  source 1..19: mol_type = other DNA
caggctggactgcggactg

SEQ ID NO: 7 - DNA, 20 bp, synthetic construct
  misc_feature 1..20: note = Synthetic oligonucleotide
  source 1..20: mol_type = other DNA
aatgcctgctccccttcacc

SEQ ID NO: 8 - DNA, 22 bp, synthetic construct
  misc_feature 1..22: note = Synthetic oligonucleotide
  source 1..22: mol_type = other DNA
ttgtctcatggttccacaagcc

SEQ ID NO: 9 - DNA, 21 bp, synthetic construct
  misc_feature 1..21: note = Synthetic oligonucleotide
  source 1..21: mol_type = other DNA
tgttaacaagagcctgggacc

SEQ ID NO: 10 - DNA, 20 bp, synthetic construct
  misc_feature 1..20: note = Synthetic oligonucleotide
  source 1..20: mol_type = other DNA
ggtgaaggggagcaggcatt

SEQ ID NO: 11 - DNA, 20 bp, synthetic construct
  misc_feature 1..20: note = Synthetic oligonucleotide
  source 1..20: mol_type = other DNA
tgtcatgagagctctgccct

SEQ ID NO: 12 - DNA, 22 bp, synthetic construct
  misc_feature 1..22: note = Synthetic oligonucleotide
  source 1..22: mol_type = other DNA
cgcctctcacgaaaactaaccc

SEQ ID NO: 13 - DNA, 20 bp, synthetic construct
  misc_feature 1..20: note = Synthetic oligonucleotide
  source 1..20: mol_type = other DNA
ggacctccctcactagcccc

SEQ ID NO: 14 - DNA, 22 bp, synthetic construct
  misc_feature 1..22: note = Synthetic oligonucleotide
  source 1..22: mol_type = other DNA
cactcatggcagaaggtgaagg

SEQ ID NO: 15 - DNA, 24 bp, synthetic construct
  misc_feature 1..24: note = Synthetic oligonucleotide
  source 1..24: mol_type = other DNA
tagatctccagcatcacatccctg

SEQ ID NO: 16 - DNA, 20 bp, synthetic construct
  misc_feature 1..20: note = Synthetic oligonucleotide
  source 1..20: mol_type = other DNA
caggaggagtggcagcaact

SEQ ID NO: 17 - DNA, 20 bp, synthetic construct
  misc_feature 1..20: note = Synthetic oligonucleotide
  source 1..20: mol_type = other DNA
cccggcagttcttccttcca

SEQ ID NO: 18 - DNA, 20 bp, synthetic construct
  misc_feature 1..20: note = Synthetic oligonucleotide
  source 1..20: mol_type = other DNA
tgaggacaaggggcacaagg

SEQ ID NO: 19 - DNA, 20 bp, synthetic construct
  misc_feature 1..20: note = Synthetic oligonucleotide
  source 1..20: mol_type = other DNA
gccccaacctgcctctaaca

SEQ ID NO: 20 - DNA, 20 bp, synthetic construct
  misc_feature 1..20: note = Synthetic oligonucleotide
  source 1..20: mol_type = other DNA
gtcctgcccagaagacagca

SEQ ID NO: 21 - DNA, 20 bp, synthetic construct
  misc_feature 1..20: note = Synthetic oligonucleotide
  source 1..20: mol_type = other DNA
ctgtggggatggggtggaag

SEQ ID NO: 22 - DNA, 20 bp, synthetic construct
  misc_feature 1..20: note = Synthetic oligonucleotide
  source 1..20: mol_type = other DNA
cccagtctcgtctcgcctac

SEQ ID NO: 23 - DNA, 20 bp, synthetic construct
  misc_feature 1..20: note = Synthetic oligonucleotide
  source 1..20: mol_type = other DNA
acccttctgccagcttgtga

SEQ ID NO: 24 - DNA, 20 bp, synthetic construct
  misc_feature 1..20: note = Synthetic oligonucleotide
  source 1..20: mol_type = other DNA
ggcccctatgtgcttgctca

SEQ ID NO: 25 - DNA, 20 bp, synthetic construct
  misc_feature 1..20: note = Synthetic oligonucleotide
  source 1..20: mol_type = other DNA
tgagcaagcacataggggcc

SEQ ID NO: 26 - DNA, 20 bp, synthetic construct
  misc_feature 1..20: note = Synthetic oligonucleotide
  source 1..20: mol_type = other DNA
gctcctgtctgccttttccg

SEQ ID NO: 27 - DNA, 20 bp, synthetic construct
  misc_feature 1..20: note = Synthetic oligonucleotide
  source 1..20: mol_type = other DNA
acacggattctggcagctgt

SEQ ID NO: 28 - DNA, 19 bp, synthetic construct
  misc_feature 1..19: note = Synthetic oligonucleotide
  source 1..19: mol_type = other DNA
gattgcagcaccccaaccc

SEQ ID NO: 29 - DNA, 20 bp, synthetic construct
  misc_feature 1..20: note = Synthetic oligonucleotide
  source 1..20: mol_type = other DNA
aagcttttgaggtgggcgtg

SEQ ID NO: 30 - DNA, 20 bp, synthetic construct
  misc_feature 1..20: note = Synthetic oligonucleotide
  source 1..20: mol_type = other DNA
atgcccatctcagcctacca

SEQ ID NO: 31 - DNA, 20 bp, synthetic construct
  misc_feature 1..20: note = Synthetic oligonucleotide
  source 1..20: mol_type = other DNA
gacatcatggggtggggagg

SEQ ID NO: 32 - DNA, 20 bp, synthetic construct
  misc_feature 1..20: note = Synthetic oligonucleotide
  source 1..20: mol_type = other DNA
tatcactgtcctcgcctgga

SEQ ID NO: 33 - DNA, 20 bp, synthetic construct
  misc_feature 1..20: note = Synthetic oligonucleotide
  source 1..20: mol_type = other DNA
tctgcaggtcctcatcagcg

SEQ ID NO: 34 - DNA, 20 bp, synthetic construct
  misc_feature 1..20: note = Synthetic oligonucleotide
  source 1..20: mol_type = other DNA
ccccactaccctgcactgag

SEQ ID NO: 35 - DNA, 20 bp, synthetic construct
  misc_feature 1..20: note = Synthetic oligonucleotide
  source 1..20: mol_type = other DNA
gtgtgttggcagtgggagga

SEQ ID NO: 36 - DNA, 20 bp, synthetic construct
  misc_feature 1..20: note = Synthetic oligonucleotide
  source 1..20: mol_type = other DNA
cctccattccaccgactccc

SEQ ID NO: 37 - DNA, 20 bp, synthetic construct
  misc_feature 1..20: note = Synthetic oligonucleotide
  source 1..20: mol_type = other DNA
gctcccttcccagatgctgt

SEQ ID NO: 38 - DNA, 20 bp, synthetic construct
  misc_feature 1..20: note = Synthetic oligonucleotide
  source 1..20: mol_type = other DNA
tggccagttgagctcaggaa

SEQ ID NO: 39 - DNA, 20 bp, synthetic construct
  misc_feature 1..20: note = Synthetic oligonucleotide
  source 1..20: mol_type = other DNA
tgtgcacggtggaaacctgt

SEQ ID NO: 40 - DNA, 20 bp, synthetic construct
  misc_feature 1..20: note = Synthetic oligonucleotide
  source 1..20: mol_type = other DNA
tcctgcaagccactacccaa

SEQ ID NO: 41 - DNA, 20 bp, synthetic construct
  misc_feature 1..20: note = Synthetic oligonucleotide
  source 1..20: mol_type = other DNA
tgttggcagtgggaggaaca

SEQ ID NO: 42 - DNA, 20 bp, synthetic construct
  misc_feature 1..20: note = Synthetic oligonucleotide
  source 1..20: mol_type = other DNA
cctcctccattccaccgact

SEQ ID NO: 43 - DNA, 21 bp, synthetic construct
  misc_feature 1..21: note = Synthetic oligonucleotide
  source 1..21: mol_type = other DNA
ggtctcgttcacctcctcacg

SEQ ID NO: 44 - DNA, 20 bp, synthetic construct
  misc_feature 1..20: note = Synthetic oligonucleotide
  source 1..20: mol_type = other DNA
cgctgatgaggacctgcaga

SEQ ID NO: 45 - DNA, 20 bp, synthetic construct
  misc_feature 1..20: note = Synthetic oligonucleotide
  source 1..20: mol_type = other DNA
gtgagcacgccattggaaca

SEQ ID NO: 46 - DNA, 20 bp, synthetic construct
  misc_feature 1..20: note = Synthetic oligonucleotide
  source 1..20: mol_type = other DNA
agcgaagtgggaaatggctg

SEQ ID NO: 47 - DNA, 19 bp, synthetic construct
  misc_feature 1..19: note = Synthetic oligonucleotide
  source 1..19: mol_type = other DNA
gggtgtgttggcagtggga

SEQ ID NO: 48 - DNA, 20 bp, synthetic construct
  misc_feature 1..20: note = Synthetic oligonucleotide
  source 1..20: mol_type = other DNA
cattccaccgactcccagca

SEQ ID NO: 49 - DNA, 20 bp, synthetic construct
  misc_feature 1..20: note = Synthetic oligonucleotide
  source 1..20: mol_type = other DNA
accagggaaaggggagcatc

SEQ ID NO: 50 - DNA, 20 bp, synthetic construct
  misc_feature 1..20: note = Synthetic oligonucleotide
  source 1..20: mol_type = other DNA
ccggggaaggaagggttagc

SEQ ID NO: 51 - DNA, 20 bp, synthetic construct
  misc_feature 1..20: note = Synthetic oligonucleotide
  source 1..20: mol_type = other DNA
gtggcaatctggtaggctgc

SEQ ID NO: 52 - DNA, 20 bp, synthetic construct
  misc_feature 1..20: note = Synthetic oligonucleotide
  source 1..20: mol_type = other DNA
cccctgtcagcgcttacact

SEQ ID NO: 53 - DNA, 20 bp, synthetic construct
  misc_feature 1..20: note = Synthetic oligonucleotide
  source 1..20: mol_type = other DNA
ctttcactttcctgccggca

SEQ ID NO: 54 - DNA, 20 bp, synthetic construct
  misc_feature 1..20: note = Synthetic oligonucleotide
  source 1..20: mol_type = other DNA
ggacagccacctacagcgaa

SEQ ID NO: 55 - DNA, 20 bp, synthetic construct
  misc_feature 1..20: note = Synthetic oligonucleotide
  source 1..20: mol_type = other DNA
gcagatttccagttgccgct

SEQ ID NO: 56 - DNA, 20 bp, synthetic construct
  misc_feature 1..20: note = Synthetic oligonucleotide
  source 1..20: mol_type = other DNA
aggccctcagactcacagtg

SEQ ID NO: 57 - DNA, 21 bp, synthetic construct
  misc_feature 1..21: note = Synthetic oligonucleotide
  source 1..21: mol_type = other DNA
tgagcacacctagccacttcc

SEQ ID NO: 58 - DNA, 20 bp, synthetic construct
  misc_feature 1..20: note = Synthetic oligonucleotide
  source 1..20: mol_type = other DNA
tcccacaccactatcctgcg

SEQ ID NO: 59 - DNA, 20 bp, synthetic construct
  misc_feature 1..20: note = Synthetic oligonucleotide
  source 1..20: mol_type = other DNA
agatgatcaacagggcccgc

SEQ ID NO: 60 - DNA, 20 bp, synthetic construct
  misc_feature 1..20: note = Synthetic oligonucleotide
  source 1..20: mol_type = other DNA
tcaggacccagatagcacgg

SEQ ID NO: 61 - DNA, 20 bp, synthetic construct
  misc_feature 1..20: note = Synthetic oligonucleotide
  source 1..20: mol_type = other DNA
acttccagggccaatgacgg

SEQ ID NO: 62 - DNA, 21 bp, synthetic construct
  misc_feature 1..21: note = Synthetic oligonucleotide
  source 1..21: mol_type = other DNA
ccaacatgtacctgtggctgc

SEQ ID NO: 63 - DNA, 20 bp, synthetic construct
  misc_feature 1..20: note = Synthetic oligonucleotide
  source 1..20: mol_type = other DNA
tcaagcagtgagaacagggc

SEQ ID NO: 64 - DNA, 20 bp, synthetic construct
  misc_feature 1..20: note = Synthetic oligonucleotide
  source 1..20: mol_type = other DNA
aaggatggggctgatggtgg

SEQ ID NO: 65 - DNA, 20 bp, synthetic construct
  misc_feature 1..20: note = Synthetic oligonucleotide
  source 1..20: mol_type = other DNA
tccacccacatccacaaccc

SEQ ID NO: 66 - DNA, 20 bp, synthetic construct
  misc_feature 1..20: note = Synthetic oligonucleotide
  source 1..20: mol_type = other DNA
tgcttctcaacagtggccga

SEQ ID NO: 67 - DNA, 20 bp, synthetic construct
  misc_feature 1..20: note = Synthetic oligonucleotide
  source 1..20: mol_type = other DNA
ctcaccctgaaccccttgca

SEQ ID NO: 68 - DNA, 20 bp, synthetic construct
  misc_feature 1..20: note = Synthetic oligonucleotide
  source 1..20: mol_type = other DNA
gcaggggtggaatggagtgt

SEQ ID NO: 69 - DNA, 20 bp, synthetic construct
  misc_feature 1..20: note = Synthetic oligonucleotide
  source 1..20: mol_type = other DNA
tgcccttcactggagagcag

SEQ ID NO: 70 - DNA, 20 bp, synthetic construct
  misc_feature 1..20: note = Synthetic oligonucleotide
  source 1..20: mol_type = other DNA
ctgctggggtttctggggaa

SEQ ID NO: 71 - DNA, 20 bp, synthetic construct
  misc_feature 1..20: note = Synthetic oligonucleotide
  source 1..20: mol_type = other DNA
ccactctcccagcctgtgac

SEQ ID NO: 72 - DNA, 20 bp, synthetic construct
  misc_feature 1..20: note = Synthetic oligonucleotide
  source 1..20: mol_type = other DNA
cgtgggtagctgtgtggaca

SEQ ID NO: 73 - DNA, 20 bp, synthetic construct
  misc_feature 1..20: note = Synthetic oligonucleotide
  source 1..20: mol_type = other DNA
tgtccacacagctacccacg

SEQ ID NO: 74 - DNA, 20 bp, synthetic construct
  misc_feature 1..20: note = Synthetic oligonucleotide
  source 1..20: mol_type = other DNA
ggcgtgtctcagtgggaaga

SEQ ID NO: 75 - DNA, 20 bp, synthetic construct
  misc_feature 1..20: note = Synthetic oligonucleotide
  source 1..20: mol_type = other DNA
ctgagtgtgtctgtgggcca

SEQ ID NO: 76 - DNA, 20 bp, synthetic construct
  misc_feature 1..20: note = Synthetic oligonucleotide
  source 1..20: mol_type = other DNA
aggacaagcagagacacgca

SEQ ID NO: 77 - DNA, 20 bp, synthetic construct
  misc_feature 1..20: note = Synthetic oligonucleotide
  source 1..20: mol_type = other DNA
gctatgttgggctggagggt

SEQ ID NO: 78 - DNA, 20 bp, synthetic construct
  misc_feature 1..20: note = Synthetic oligonucleotide
  source 1..20: mol_type = other DNA
gagcgccacatgtcctctga

SEQ ID NO: 79 - DNA, 20 bp, synthetic construct
  misc_feature 1..20: note = Synthetic oligonucleotide
  source 1..20: mol_type = other DNA
cctgggaccctgagttgcaa

SEQ ID NO: 80 - DNA, 20 bp, synthetic construct
  misc_feature 1..20: note = Synthetic oligonucleotide
  source 1..20: mol_type = other DNA
ccatgggcctgagtcactcc

SEQ ID NO: 81 - DNA, 20 bp, synthetic construct
  misc_feature 1..20: note = Synthetic oligonucleotide
  source 1..20: mol_type = other DNA
tttcctctctcccgccctct

SEQ ID NO: 82 - DNA, 20 bp, synthetic construct
  misc_feature 1..20: note = Synthetic oligonucleotide
  source 1..20: mol_type = other DNA
tgcgggagtttgggaccttt

SEQ ID NO: 83 - DNA, 20 bp, synthetic construct
  misc_feature 1..20: note = Synthetic oligonucleotide
  source 1..20: mol_type = other DNA
aggcttgcctgggaagtgaa

SEQ ID NO: 84 - DNA, 20 bp, synthetic construct
  misc_feature 1..20: note = Synthetic oligonucleotide
  source 1..20: mol_type = other DNA
cctggggtggtgctttgaga

SEQ ID NO: 85 - DNA, 20 bp, synthetic construct
  misc_feature 1..20: note = Synthetic oligonucleotide
  source 1..20: mol_type = other DNA
tccccgcccaaatctcatgt

SEQ ID NO: 86 - DNA, 20 bp, synthetic construct
  misc_feature 1..20: note = Synthetic oligonucleotide
  source 1..20: mol_type = other DNA
acccaaacaccctccaccag

SEQ ID NO: 87 - DNA, 23 bp, synthetic construct
  misc_feature 1..23: note = Synthetic oligonucleotide
  source 1..23: mol_type = other DNA
gaaagccctctctgtgcctgaat

SEQ ID NO: 88 - DNA, 21 bp, synthetic construct
  misc_feature 1..21: note = Synthetic oligonucleotide
  source 1..21: mol_type = other DNA
agaactgctctcggacaaaca

SEQ ID NO: 89 - DNA, 20 bp, synthetic construct
  misc_feature 1..20: note = Synthetic oligonucleotide
  source 1..20: mol_type = other DNA
aagcggcacagaaacatcgg

SEQ ID NO: 90 - DNA, 20 bp, synthetic construct
  misc_feature 1..20: note = Synthetic oligonucleotide
  source 1..20: mol_type = other DNA
cccagcccagcctacttctt

SEQ ID NO: 91 - DNA, 20 bp, synthetic construct
  misc_feature 1..20: note = Synthetic oligonucleotide
  source 1..20: mol_type = other DNA
cagctacgtgactcagggca

SEQ ID NO: 92 - DNA, 21 bp, synthetic construct
  misc_feature 1..21: note = Synthetic oligonucleotide
  source 1..21: mol_type = other DNA
tgcctcccatcttgccaatga

SEQ ID NO: 93 - DNA, 20 bp, synthetic construct
  misc_feature 1..20: note = Synthetic oligonucleotide
  source 1..20: mol_type = other DNA
cagaccgagggctccaacac

SEQ ID NO: 94 - DNA, 20 bp, synthetic construct
  misc_feature 1..20: note = Synthetic oligonucleotide
  source 1..20: mol_type = other DNA
tctctctgggaaaacgcggt

SEQ ID NO: 95 - DNA, 20 bp, synthetic construct
  misc_feature 1..20: note = Synthetic oligonucleotide
  source 1..20: mol_type = other DNA
gagcagagtgaaggggcagt

SEQ ID NO: 96 - DNA, 19 bp, synthetic construct
  misc_feature 1..19: note = Synthetic oligonucleotide
  source 1..19: mol_type = other DNA
cctggtggtctggtctgcc

SEQ ID NO: 97 - DNA, 20 bp, synthetic construct
  misc_feature 1..20: note = Synthetic oligonucleotide
  source 1..20: mol_type = other DNA
tcactgggcaaggaagaggc

SEQ ID NO: 98 - DNA, 20 bp, synthetic construct
  misc_feature 1..20: note = Synthetic oligonucleotide
  source 1..20: mol_type = other DNA
ccttctgtctcctgagcccc

SEQ ID NO: 99 - DNA, 20 bp, synthetic construct
  misc_feature 1..20: note = Synthetic oligonucleotide
  source 1..20: mol_type = other DNA
caagcaccgcgttttcccag

SEQ ID NO: 100 - DNA, 20 bp, synthetic construct
  misc_feature 1..20: note = Synthetic oligonucleotide
  source 1..20: mol_type = other DNA
cctggggtggtgctttgaga

SEQ ID NO: 101 - DNA, 20 bp, synthetic construct
  misc_feature 1..20: note = Synthetic oligonucleotide
  source 1..20: mol_type = other DNA
gcaaggaagaggccaagggt

SEQ ID NO: 102 - DNA, 20 bp, synthetic construct
  misc_feature 1..20: note = Synthetic oligonucleotide
  source 1..20: mol_type = other DNA
ggcccactgtcccttctgtc

SEQ ID NO: 103 - DNA, 20 bp, synthetic construct
  misc_feature 1..20: note = Synthetic oligonucleotide
  source 1..20: mol_type = other DNA
tcggaaacagccagaggagg

SEQ ID NO: 104 - DNA, 20 bp, synthetic construct
  misc_feature 1..20: note = Synthetic oligonucleotide
  source 1..20: mol_type = other DNA
actcggatggcagggtgaat

SEQ ID NO: 105 - DNA, 20 bp, synthetic construct
  misc_feature 1..20: note = Synthetic oligonucleotide
  source 1..20: mol_type = other DNA
aggcttgcctgggaagtgaa

SEQ ID NO: 106 - DNA, 21 bp, synthetic construct
  misc_feature 1..21: note = Synthetic oligonucleotide
  source 1..21: mol_type = other DNA
cgggttcttagcgtcctcact

SEQ ID NO: 107 - DNA, 21 bp, synthetic construct
  misc_feature 1..21: note = Synthetic oligonucleotide
  source 1..21: mol_type = other DNA
tgggaggtggcatttgagagg

SEQ ID NO: 108 - DNA, 20 bp, synthetic construct
  misc_feature 1..20: note = Synthetic oligonucleotide
  source 1..20: mol_type = other DNA
ccctctgccaccatttcagc

SEQ ID NO: 109 - DNA, 20 bp, synthetic construct
  misc_feature 1..20: note = Synthetic oligonucleotide
  source 1..20: mol_type = other DNA
agaagaagcaccgcacgagt

SEQ ID NO: 110 - DNA, 21 bp, synthetic construct
  misc_feature 1..21: note = Synthetic oligonucleotide
  source 1..21: mol_type = other DNA
gggacatttcagactggcacc

SEQ ID NO: 111 - DNA, 20 bp, synthetic construct
  misc_feature 1..20: note = Synthetic oligonucleotide
  source 1..20: mol_type = other DNA
tgcccaacccatttctccct

SEQ ID NO: 112 - DNA, 20 bp, synthetic construct
  misc_feature 1..20: note = Synthetic oligonucleotide
  source 1..20: mol_type = other DNA
tggattctgtgggcttgcag

SEQ ID NO: 113 - DNA, 20 bp, synthetic construct
  misc_feature 1..20: note = Synthetic oligonucleotide
  source 1..20: mol_type = other DNA
tccaccccactctgaggtca

SEQ ID NO: 114 - DNA, 20 bp, synthetic construct
  misc_feature 1..20: note = Synthetic oligonucleotide
  source 1..20: mol_type = other DNA
gaggtgggagtgggattcgg

SEQ ID NO: 115 - DNA, 26 bp, synthetic construct
  misc_feature 1..26: note = Synthetic oligonucleotide
  source 1..26: mol_type = other DNA
gtgaacctagcgtcatacagcctaag

SEQ ID NO: 116 - DNA, 24 bp, synthetic construct
  misc_feature 1..24: note = Synthetic oligonucleotide
  source 1..24: mol_type = other DNA
ttgacttgccttatctgatccccg

SEQ ID NO: 117 - DNA, 20 bp, synthetic construct
  misc_feature 1..20: note = Synthetic oligonucleotide
  source 1..20: mol_type = other DNA
aaacacacagggccgaggaa

SEQ ID NO: 118 - DNA, 20 bp, synthetic construct
  misc_feature 1..20: note = Synthetic oligonucleotide
  source 1..20: mol_type = other DNA
aagtgactggcctcctgagc

SEQ ID NO: 119 - DNA, 20 bp, synthetic construct
  misc_feature 1..20: note = Synthetic oligonucleotide
  source 1..20: mol_type = other DNA
ccacttgtccctaccccacc

SEQ ID NO: 120 - DNA, 20 bp, synthetic construct
  misc_feature 1..20: note = Synthetic oligonucleotide
  source 1..20: mol_type = other DNA
acttaacaggtcgcgctggt

SEQ ID NO: 121 - DNA, 20 bp, synthetic construct
  misc_feature 1..20: note = Synthetic oligonucleotide
  source 1..20: mol_type = other DNA
gcacaaccgcacacccatac

SEQ ID NO: 122 - DNA, 20 bp, synthetic construct
  misc_feature 1..20: note = Synthetic oligonucleotide
  source 1..20: mol_type = other DNA
cgtgggtagctgtgtggaca

SEQ ID NO: 123 - DNA, 20 bp, synthetic construct
  misc_feature 1..20: note = Synthetic oligonucleotide
  source 1..20: mol_type = other DNA
ctcctccacctgctgttccc

SEQ ID NO: 124 - DNA, 20 bp, synthetic construct
  misc_feature 1..20: note = Synthetic oligonucleotide
  source 1..20: mol_type = other DNA
tgcaggcgtgtaaatgtggc

SEQ ID NO: 125 - DNA, 20 bp, synthetic construct
  misc_feature 1..20: note = Synthetic oligonucleotide
  source 1..20: mol_type = other DNA
ctgcacgccactcaacactc

SEQ ID NO: 126 - DNA, 20 bp, synthetic construct
  misc_feature 1..20: note = Synthetic oligonucleotide
  source 1..20: mol_type = other DNA
gggaacagcaggtggaggag

SEQ ID NO: 127 - DNA, 20 bp, synthetic construct
  misc_feature 1..20: note = Synthetic oligonucleotide
  source 1..20: mol_type = other DNA
atggaggcttggctgtgagg

SEQ ID NO: 128 - DNA, 20 bp, synthetic construct
  misc_feature 1..20: note = Synthetic oligonucleotide
  source 1..20: mol_type = other DNA
agaagacgcagcgcttggta

SEQ ID NO: 129 - DNA, 21 bp, synthetic construct
  misc_feature 1..21: note = Synthetic oligonucleotide
  source 1..21: mol_type = other DNA
agctctgccctcatgaatgct

SEQ ID NO: 130 - DNA, 22 bp, synthetic construct
  misc_feature 1..22: note = Synthetic oligonucleotide
  source 1..22: mol_type = other DNA
accctcctgtactcctttgtcc

SEQ ID NO: 131 - DNA, 22 bp, synthetic construct
  misc_feature 1..22: note = Synthetic oligonucleotide
  source 1..22: mol_type = other DNA
agaggggtgatagctaaagggt

SEQ ID NO: 132 - DNA, 20 bp, synthetic construct
  misc_feature 1..20: note = Synthetic oligonucleotide
  source 1..20: mol_type = other DNA
ggtgggttgaggggctagtg

SEQ ID NO: 133 - DNA, 21 bp, synthetic construct
  misc_feature 1..21: note = Synthetic oligonucleotide
  source 1..21: mol_type = other DNA
tcttgtctcccatctgccaca

SEQ ID NO: 134 - DNA, 22 bp, synthetic construct
  misc_feature 1..22: note = Synthetic oligonucleotide
  source 1..22: mol_type = other DNA
tgtacagggatgtgatgctgga

SEQ ID NO: 135 - DNA, 20 bp, synthetic construct
  misc_feature 1..20: note = Synthetic oligonucleotide
  source 1..20: mol_type = other DNA
gatggcaatctgggtggaga

SEQ ID NO: 136 - DNA, 22 bp, synthetic construct
  misc_feature 1..22: note = Synthetic oligonucleotide
  source 1..22: mol_type = other DNA
ttgtccaatccagtgcctctcc

SEQ ID NO: 137 - DNA, 24 bp, synthetic construct
  misc_feature 1..24: note = Synthetic oligonucleotide
  source 1..24: mol_type = other DNA
gggtgatagctaaagggtacaggg

SEQ ID NO: 138 - DNA, 20 bp, synthetic construct
  misc_feature 1..20: note = Synthetic oligonucleotide
  source 1..20: mol_type = other DNA
atatggtgggttgaggggct

SEQ ID NO: 139 - DNA, 21 bp, synthetic construct
  misc_feature 1..21: note = Synthetic oligonucleotide
  source 1..21: mol_type = other DNA
aggtgggacttagtgggaggt

SEQ ID NO: 140 - DNA, 24 bp, synthetic construct
  misc_feature 1..24: note = Synthetic oligonucleotide
  source 1..24: mol_type = other DNA
tcgctaggcttacttgacttcagt

SEQ ID NO: 141 - DNA, 22 bp, synthetic construct
  misc_feature 1..22: note = Synthetic oligonucleotide
  source 1..22: mol_type = other DNA
ccatggctcttctccttgttcc

SEQ ID NO: 142 - DNA, 20 bp, synthetic construct
  misc_feature 1..20: note = Synthetic oligonucleotide
  source 1..20: mol_type = other DNA
tttgaggatgtggctgtgga

SEQ ID NO: 143 - DNA, 24 bp, synthetic construct
  misc_feature 1..24: note = Synthetic oligonucleotide
  source 1..24: mol_type = other DNA
gctaaataatgccagtctgccagc

SEQ ID NO: 144 - DNA, 21 bp, synthetic construct
  misc_feature 1..21: note = Synthetic oligonucleotide
  source 1..21: mol_type = other DNA
tcttgaatggcagcagtgtcg

SEQ ID NO: 145 - DNA, 20 bp, synthetic construct
  misc_feature 1..20: note = Synthetic oligonucleotide
  source 1..20: mol_type = other DNA
aaccgtggcattggaaggga

SEQ ID NO: 146 - DNA, 20 bp, synthetic construct
  misc_feature 1..20: note = Synthetic oligonucleotide
  source 1..20: mol_type = other DNA
gggtgtgactgagagggagc

SEQ ID NO: 147 - DNA, 20 bp, synthetic construct
  misc_feature 1..20: note = Synthetic oligonucleotide
  source 1..20: mol_type = other DNA
tgggagtaggcgagacgaga

SEQ ID NO: 148 - DNA, 20 bp, synthetic construct
  misc_feature 1..20: note = Synthetic oligonucleotide
  source 1..20: mol_type = other DNA
tggcagaagggtgggctttt

SEQ ID NO: 149 - DNA, 20 bp, synthetic construct
  misc_feature 1..20: note = Synthetic oligonucleotide
  source 1..20: mol_type = other DNA
cacacacacacacacccacg

SEQ ID NO: 150 - DNA, 20 bp, synthetic construct
  misc_feature 1..20: note = Synthetic oligonucleotide
  source 1..20: mol_type = other DNA
tgtccgcagagcacaagagg

SEQ ID NO: 151 - DNA, 20 bp, synthetic construct
  misc_feature 1..20: note = Synthetic oligonucleotide
  source 1..20: mol_type = other DNA
gtaggcgagacgagactggg

SEQ ID NO: 152 - DNA, 20 bp, synthetic construct
  misc_feature 1..20: note = Synthetic oligonucleotide
  source 1..20: mol_type = other DNA
tcacaagctggcagaagggt

SEQ ID NO: 153 - DNA, 20 bp, synthetic construct
  misc_feature 1..20: note = Synthetic oligonucleotide
  source 1..20: mol_type = other DNA
ttgagattggcgtggggtca

SEQ ID NO: 154 - DNA, 20 bp, synthetic construct
  misc_feature 1..20: note = Synthetic oligonucleotide
  source 1..20: mol_type = other DNA
cactccagaggcacacaggg

SEQ ID NO: 155 - DNA, 20 bp, synthetic construct
  misc_feature 1..20: note = Synthetic oligonucleotide
  source 1..20: mol_type = other DNA
ttggggcagtggtaggtgag

SEQ ID NO: 156 - DNA, 20 bp, synthetic construct
  misc_feature 1..20: note = Synthetic oligonucleotide
  source 1..20: mol_type = other DNA
atcggattgcagcaccccaa

SEQ ID NO: 157 - DNA, 20 bp, synthetic construct
  misc_feature 1..20: note = Synthetic oligonucleotide
  source 1..20: mol_type = other DNA
tgcccagattcccaccttca

SEQ ID NO: 158 - DNA, 20 bp, synthetic construct
  misc_feature 1..20: note = Synthetic oligonucleotide
  source 1..20: mol_type = other DNA
ctcacctcccagcttccacc

SEQ ID NO: 159 - DNA, 20 bp, synthetic construct
  misc_feature 1..20: note = Synthetic oligonucleotide
  source 1..20: mol_type = other DNA
gctgtcatggagcgctgtct

SEQ ID NO: 160 - DNA, 20 bp, synthetic construct
  misc_feature 1..20: note = Synthetic oligonucleotide
  source 1..20: mol_type = other DNA
cccagtctcgtctcgcctac

SEQ ID NO: 161 - DNA, 20 bp, synthetic construct
  misc_feature 1..20: note = Synthetic oligonucleotide
  source 1..20: mol_type = other DNA
ctggctctggatggcttgga

SEQ ID NO: 162 - DNA, 20 bp, synthetic construct
  misc_feature 1..20: note = Synthetic oligonucleotide
  source 1..20: mol_type = other DNA
caccctgtgttccaatggcg

SEQ ID NO: 163 - DNA, 20 bp, synthetic construct
  misc_feature 1..20: note = Synthetic oligonucleotide
  source 1..20: mol_type = other DNA
gggctgatgtggctagggat

SEQ ID NO: 164 - DNA, 20 bp, synthetic construct
  misc_feature 1..20: note = Synthetic oligonucleotide
  source 1..20: mol_type = other DNA
cctccattccaccgactccc

SEQ ID NO: 165 - DNA, 20 bp, synthetic construct
  misc_feature 1..20: note = Synthetic oligonucleotide
  source 1..20: mol_type = other DNA
ggatctggctctggatggct

SEQ ID NO: 166 - DNA, 20 bp, synthetic construct
  misc_feature 1..20: note = Synthetic oligonucleotide
  source 1..20: mol_type = other DNA
cctgtgttccaatggcgtgc

SEQ ID NO: 167 - DNA, 20 bp, synthetic construct
  misc_feature 1..20: note = Synthetic oligonucleotide
  source 1..20: mol_type = other DNA
gtgagcacgccattggaaca

SEQ ID NO: 168 - DNA, 20 bp, synthetic construct
  misc_feature 1..20: note = Synthetic oligonucleotide
  source 1..20: mol_type = other DNA
tcctgcaagccactacccaa

SEQ ID NO: 169 - DNA, 20 bp, synthetic construct
  misc_feature 1..20: note = Synthetic oligonucleotide
  source 1..20: mol_type = other DNA
acgtcgtggcttcaaagtgc

SEQ ID NO: 170 - DNA, 20 bp, synthetic construct
  misc_feature 1..20: note = Synthetic oligonucleotide
  source 1..20: mol_type = other DNA
agcgaagtgggaaatggctg

SEQ ID NO: 171 - DNA, 20 bp, synthetic construct
  misc_feature 1..20: note = Synthetic oligonucleotide
  source 1..20: mol_type = other DNA
catctcgggccatgacgtcc

SEQ ID NO: 172 - DNA, 20 bp, synthetic construct
  misc_feature 1..20: note = Synthetic oligonucleotide
  source 1..20: mol_type = other DNA
tctggagctggatgactggc

SEQ ID NO: 173 - DNA, 20 bp, synthetic construct
  misc_feature 1..20: note = Synthetic oligonucleotide
  source 1..20: mol_type = other DNA
ggtcgggctggtctcaaact

SEQ ID NO: 174 - DNA, 20 bp, synthetic construct
  misc_feature 1..20: note = Synthetic oligonucleotide
  source 1..20: mol_type = other DNA
gcaatatgaggctgggcaca

SEQ ID NO: 175 - DNA, 19 bp, synthetic construct
  misc_feature 1..19: note = Synthetic oligonucleotide
  source 1..19: mol_type = other DNA
gcccggtgtccatgtcctt

SEQ ID NO: 176 - DNA, 20 bp, synthetic construct
  misc_feature 1..20: note = Synthetic oligonucleotide
  source 1..20: mol_type = other DNA
tcctcccactgccaacacac

SEQ ID NO: 177 - DNA, 20 bp, synthetic construct
  misc_feature 1..20: note = Synthetic oligonucleotide
  source 1..20: mol_type = other DNA
gatccacccacctcagcctc

SEQ ID NO: 178 - DNA, 20 bp, synthetic construct
  misc_feature 1..20: note = Synthetic oligonucleotide
  source 1..20: mol_type = other DNA
ccgtcattggccctggaagt

SEQ ID NO: 179 - DNA, 20 bp, synthetic construct
  misc_feature 1..20: note = Synthetic oligonucleotide
  source 1..20: mol_type = other DNA
acttccagggccaatgacgg

SEQ ID NO: 180 - DNA, 20 bp, synthetic construct
  misc_feature 1..20: note = Synthetic oligonucleotide
  source 1..20: mol_type = other DNA
aattccccaagccagccact

SEQ ID NO: 181 - DNA, 20 bp, synthetic construct
  misc_feature 1..20: note = Synthetic oligonucleotide
  source 1..20: mol_type = other DNA
ccacctcagcctcccaaagt

SEQ ID NO: 182 - DNA, 20 bp, synthetic construct
  misc_feature 1..20: note = Synthetic oligonucleotide
  source 1..20: mol_type = other DNA
agtcctacccgtcattggcc

SEQ ID NO: 183 - DNA, 21 bp, synthetic construct
  misc_feature 1..21: note = Synthetic oligonucleotide
  source 1..21: mol_type = other DNA
aggttgtcgatgaactgggca

SEQ ID NO: 184 - DNA, 20 bp, synthetic construct
  misc_feature 1..20: note = Synthetic oligonucleotide
  source 1..20: mol_type = other DNA
cacacagccacacagccatc

SEQ ID NO: 185 - DNA, 20 bp, synthetic construct
  misc_feature 1..20: note = Synthetic oligonucleotide
  source 1..20: mol_type = other DNA
ccgcacacatgtcagggaga

SEQ ID NO: 186 - DNA, 21 bp, synthetic construct
  misc_feature 1..21: note = Synthetic oligonucleotide
  source 1..21: mol_type = other DNA
acaacttggaggctcaggacc

SEQ ID NO: 187 - DNA, 20 bp, synthetic construct
  misc_feature 1..20: note = Synthetic oligonucleotide
  source 1..20: mol_type = other DNA
ggtgagggtgggatgtgtca

SEQ ID NO: 188 - DNA, 20 bp, synthetic construct
  misc_feature 1..20: note = Synthetic oligonucleotide
  source 1..20: mol_type = other DNA
ttagcctgacgtgccatgag

SEQ ID NO: 189 - DNA, 19 bp, synthetic construct
  misc_feature 1..19: note = Synthetic oligonucleotide
  source 1..19: mol_type = other DNA
acccacctcagcctcccaa

SEQ ID NO: 190 - DNA, 20 bp, synthetic construct
  misc_feature 1..20: note = Synthetic oligonucleotide
  source 1..20: mol_type = other DNA
ctacccgtcattggccctgg

SEQ ID NO: 191 - DNA, 20 bp, synthetic construct
  misc_feature 1..20: note = Synthetic oligonucleotide
  source 1..20: mol_type = other DNA
ctggcccactacctcccaag

SEQ ID NO: 192 - DNA, 18 bp, synthetic construct
  misc_feature 1..18: note = Synthetic oligonucleotide
  source 1..18: mol_type = other DNA
cctgctcaacgtggccct